European Patent Specification EP 3 610 035 B1, published June 5, 2024. Title: COMPOSITIONS AND METHODS FOR TRANSIENT GENE THERAPY WITH ENHANCED STABILITY. Applicant: Dana-Farber Cancer Institute, Inc. Application Not Yet Assigned. The sequence listing filed with the application follows.

SEQUENCE LISTING (93 sequences)

SEQ ID NO: 1 - DNA, 30 bp, Artificial Sequence
  Synthetic polynucleotide
gcacgaattgcacaatcggtacgttcgagt

SEQ ID NO: 2 - DNA, 30 bp, Artificial Sequence
  Synthetic polynucleotide
gttacgtaccaacacgttattgccgtcggt

SEQ ID NO: 3 - DNA, 20 bp, Artificial Sequence
  Synthetic polynucleotide
gcacgaattgcacaatcggt

SEQ ID NO: 4 - DNA, 20 bp, Artificial Sequence
  Synthetic polynucleotide
tggctgcacgaattgcacaa

SEQ ID NO: 5 - DNA, 20 bp, Artificial Sequence
  Synthetic polynucleotide
gtacgtggctgcacgaattg

SEQ ID NO: 6 - DNA, 15 bp, Artificial Sequence
  Synthetic polynucleotide
gcacgaattgcacaa

SEQ ID NO: 7 - DNA, 15 bp, Artificial Sequence
  Synthetic polynucleotide
tggctgcacgaattg

SEQ ID NO: 8 - DNA, 30 bp, Artificial Sequence
  Synthetic polynucleotide
actcgaaagaacagaatgtacaaatcgtgc

SEQ ID NO: 9 - DNA, 30 bp, Artificial Sequence
  Synthetic polynucleotide
accgaaggcattaaagtgatggaacataac

SEQ ID NO: 10 - DNA, 30 bp, Artificial Sequence
  Synthetic polynucleotide
accgtcggaaatgacgtattgattcgtaac

SEQ ID NO: 11 - DNA, 30 bp, Artificial Sequence
  Synthetic polynucleotide
accgtcggaaatgacgtattgataggtaac

SEQ ID NO: 12 - DNA, 30 bp, Artificial Sequence
  Synthetic polynucleotide
actcaaaagtaacgaatgtgaaattagtgc

SEQ ID NO: 13 - DNA, 30 bp, Artificial Sequence
  Synthetic polynucleotide
accgacagcaacaacctgctggtacataac

SEQ ID NO: 14 - DNA, 30 bp, Artificial Sequence
  Synthetic polynucleotide
actcaagcgtactgagtgtggaactagtgc

SEQ ID NO: 15 - DNA, 30 bp, Artificial Sequence
  Synthetic polynucleotide
accgccggaaatgacgtattgataggtaac

SEQ ID NO: 16 - DNA, 30 bp, Artificial Sequence
  Synthetic polynucleotide
accgtcggaaattaagtattgatacgtaac

SEQ ID NO: 17 - DNA, 30 bp, Artificial Sequence
  Synthetic polynucleotide
actcaaacataacgatagtgcaaatagtgc

SEQ ID NO: 18 - DNA, 30 bp, Artificial Sequence
  Synthetic polynucleotide
actcaagcgtacggaatgtggaaatggtgc

SEQ ID NO: 19 - DNA, 30 bp, Artificial Sequence
  Synthetic polynucleotide
actccaacatacagatagtgcaaatagtgc

SEQ ID NO: 20 - DNA, 30 bp, Artificial Sequence
  Synthetic polynucleotide
accgccggaaatcacgtattgataggtaac

SEQ ID NO: 21 - DNA, 30 bp, Artificial Sequence
  Synthetic polynucleotide
actcaaacatacagatagtgcaaatagtgc

SEQ ID NO: 22 - DNA, 30 bp, Artificial Sequence
  Synthetic polynucleotide
accgacagcaacaacttgctgctatgtaac

SEQ ID NO: 23 - DNA, 30 bp, Artificial Sequence
  Synthetic polynucleotide
actcaaaagtaacgaatgtgaaaatagtgc

SEQ ID NO: 24 - DNA, 30 bp, Artificial Sequence
  Synthetic polynucleotide
accgacagcaacaacctgctgctatgtaac

SEQ ID NO: 25 - DNA, 20 bp, Artificial Sequence
  Synthetic polynucleotide
accgattgagctatacgtgc

SEQ ID NO: 26 - DNA, 20 bp, Artificial Sequence
  Synthetic polynucleotide
ttgtacaattcatgcagcca

SEQ ID NO: 27 - DNA, 20 bp, Artificial Sequence
  Synthetic polynucleotide
accgattgtccaatccgtgc

SEQ ID NO: 28 - DNA, 20 bp, Artificial Sequence
  Synthetic polynucleotide
ttgtggaatccgtggagcca

SEQ ID NO: 29 - DNA, 20 bp, Artificial Sequence
  Synthetic polynucleotide
caatacgtgccgccaggtac

SEQ ID NO: 30 - DNA, 20 bp, Artificial Sequence
  Synthetic polynucleotide
accggttgtgaaattggtgc

SEQ ID NO: 31 - DNA, 20 bp, Artificial Sequence
  Synthetic polynucleotide
ttgtccaattcctgcagcca

SEQ ID NO: 32 - DNA, 20 bp, Artificial Sequence
  Synthetic polynucleotide
accgcttatgcagttcgtgc

SEQ ID NO: 33 - DNA, 20 bp, Artificial Sequence
  Synthetic polynucleotide
caattagtgaagcctcgtac

SEQ ID NO: 34 - DNA, 20 bp, Artificial Sequence
  Synthetic polynucleotide
accgactgtgccattggtgc

SEQ ID NO: 35 - DNA, 20 bp, Artificial Sequence
  Synthetic polynucleotide
accgtttgttcaatttgtgc

SEQ ID NO: 36 - DNA, 20 bp, Artificial Sequence
  Synthetic polynucleotide
accggttgtacaatccgtgc

SEQ ID NO: 37 - DNA, 20 bp, Artificial Sequence
  Synthetic polynucleotide
accggttgtccaatccgtgc

SEQ ID NO: 38 - DNA, 20 bp, Artificial Sequence
  Synthetic polynucleotide
accgaatgagctatacgtgc

SEQ ID NO: 39 - DNA, 20 bp, Artificial Sequence
  Synthetic polynucleotide
caattcatgcatccaggtac

SEQ ID NO: 40 - DNA, 20 bp, Artificial Sequence
  Synthetic polynucleotide
ttgtacacttcatgcagcca

SEQ ID NO: 41 - DNA, 20 bp, Artificial Sequence
  Synthetic polynucleotide
caatacgtggagacaagtac

SEQ ID NO: 42 - DNA, 15 bp, Artificial Sequence
  Synthetic polynucleotide
ttgtccaattcgtgc

SEQ ID NO: 43 - DNA, 15 bp, Artificial Sequence
  Synthetic polynucleotide
caatacgtgcagcca

SEQ ID NO: 44 - DNA, 15 bp, Artificial Sequence
  Synthetic polynucleotide
ttgtgcaatgcgtgc

SEQ ID NO: 45 - DNA, 15 bp, Artificial Sequence
  Synthetic polynucleotide
caattcgagcagcca

SEQ ID NO: 46 - DNA, 15 bp, Artificial Sequence
  Synthetic polynucleotide
ttgtggaattcgtgc

SEQ ID NO: 47 - DNA, 15 bp, Artificial Sequence
  Synthetic polynucleotide
ttgtgcaatacgtgc

SEQ ID NO: 48 - DNA, 15 bp, Artificial Sequence
  Synthetic polynucleotide
ttgtgcaaatcgtgc

SEQ ID NO: 49 - DNA, 15 bp, Artificial Sequence
  Synthetic polynucleotide
caattagtgcagcca

SEQ ID NO: 50 - DNA, 15 bp, Artificial Sequence
  Synthetic polynucleotide
caattcgtgaagcca

SEQ ID NO: 51 - DNA, 15 bp, Artificial Sequence
  Synthetic polynucleotide
caatccgtgcagcca

SEQ ID NO: 52 - DNA, 15 bp, Artificial Sequence
  Synthetic polynucleotide
ttgtgcaattagtgc

SEQ ID NO: 53 - DNA, 15 bp, Artificial Sequence
  Synthetic polynucleotide
ttgtgcgagtcgtgc

SEQ ID NO: 54 - DNA, 15 bp, Artificial Sequence
  Synthetic polynucleotide
caattcgtacagcca

SEQ ID NO: 55 - DNA, 15 bp, Artificial Sequence
  Synthetic polynucleotide
ttgtgctagtcgtgc

SEQ ID NO: 56 - DNA, 15 bp, Artificial Sequence
  Synthetic polynucleotide
caattcgagctgcca

SEQ ID NO: 57 - DNA, 15 bp, Artificial Sequence
  Synthetic polynucleotide
caattcgcgctgcca

SEQ ID NO: 58 - DNA, 10 bp, Artificial Sequence
  Synthetic polynucleotide
gggaatcgac

SEQ ID NO: 59 - DNA, 10 bp, Artificial Sequence
  Synthetic polynucleotide
gggaaaaaaa

SEQ ID NO: 60 - DNA, 10 bp, Artificial Sequence
  Synthetic polynucleotide
ggaaaaaaaa

SEQ ID NO: 61 - DNA, 10 bp, Artificial Sequence
  Synthetic polynucleotide
gaaaaaaaaa

SEQ ID NO: 62 - DNA, 10 bp, Artificial Sequence
  Synthetic polynucleotide
gccccccccc

SEQ ID NO: 63 - DNA, 15 bp, Artificial Sequence
  Synthetic polynucleotide
gggaatcgactacag

SEQ ID NO: 64 - DNA, 15 bp, Artificial Sequence
  Synthetic polynucleotide
gggaaaaaaaaaaaa

SEQ ID NO: 65 - DNA, 15 bp, Artificial Sequence
  Synthetic polynucleotide
ggaaaaaaaaaaaaa

SEQ ID NO: 66 - DNA, 15 bp, Artificial Sequence
  Synthetic polynucleotide
gaaaaaaaaaaaaaa

SEQ ID NO: 67 - DNA, 15 bp, Artificial Sequence
  Synthetic polynucleotide
gcccccccccccccc

SEQ ID NO: 68 - DNA, 20 bp, Artificial Sequence
  Synthetic polynucleotide
gggaatcgactacaggagga

SEQ ID NO: 69 - DNA, 20 bp, Artificial Sequence
  Synthetic polynucleotide
gggaaaaaaaaaaaaaaaaa

SEQ ID NO: 70 - DNA, 10 bp, Artificial Sequence
  Synthetic polynucleotide
cggaatatag

SEQ ID NO: 71 - DNA, 10 bp, Artificial Sequence
  Synthetic polynucleotide
aaaaaaaaaa

SEQ ID NO: 72 - DNA, 10 bp, Artificial Sequence
  Synthetic polynucleotide
cccccccccc

SEQ ID NO: 73 - DNA, 15 bp, Artificial Sequence
  Synthetic polynucleotide
cggaatatagaagca

SEQ ID NO: 74 - DNA, 15 bp, Artificial Sequence
  Synthetic polynucleotide
aaaaaaaaaaaaaaa

SEQ ID NO: 75 - DNA, 15 bp, Artificial Sequence
  Synthetic polynucleotide
ccccccccccccccc

SEQ ID NO: 76 - DNA, 20 bp, Artificial Sequence
  Synthetic polynucleotide
cggaatatagaagcataaga

SEQ ID NO: 77 - DNA, 20 bp, Artificial Sequence
  Synthetic polynucleotide
aaaaaaaaaaaaaaaaaaaa

SEQ ID NO: 78 - DNA, 20 bp, Artificial Sequence
  Synthetic polynucleotide
cccccccccccccccccccc

SEQ ID NO: 79 - DNA, 50 bp, Artificial Sequence
  Synthetic polynucleotide
taatacgactcactatagggttatgataactggctgcacgaattgcacaa

SEQ ID NO: 80 - DNA, 30 bp, Artificial Sequence
  Synthetic polynucleotide
agcgacttcgttgtgcaattcgtgcagcca

SEQ ID NO: 81 - DNA, 10 bp, Artificial Sequence
  Synthetic polynucleotide
tgccgtcggt

SEQ ID NO: 82 - DNA, 10 bp, Artificial Sequence
  Synthetic polynucleotide
accgacggca

SEQ ID NO: 83 - DNA, 50 bp, Artificial Sequence
  Synthetic polynucleotide
aaaaaaaaaaaaaaaaaaaaaaaaaaaaaaaccgacggcaaaaaaaaaaa

SEQ ID NO: 84 - DNA, 50 bp, Artificial Sequence
  Synthetic polynucleotide
tttttttttttttttttttttttttttttttggctgccgttttttttttt

SEQ ID NO: 85 - DNA, 50 bp, Artificial Sequence
  Synthetic polynucleotide
gggaaaaaaatgccgtcggtacgttactggccgaagccgcttggaataag

SEQ ID NO: 86 - DNA, 50 bp, Artificial Sequence
  Synthetic polynucleotide
ccctttttttacggcagccatgcaatgaccggcttcggcgaaccttattc

SEQ ID NO: 87 - DNA, 10 bp, Artificial Sequence
  Synthetic polynucleotide
gcacgaattg

SEQ ID NO: 88 - DNA, 30 bp, Artificial Sequence
  Synthetic polynucleotide
actcgaacgtaccgattgtgcaattcgtgc

SEQ ID NO: 89 - DNA, 20 bp, Artificial Sequence
  Synthetic polynucleotide
accgattgtgcaattcgtgc

SEQ ID NO: 90 - DNA, 15 bp, Artificial Sequence
  Synthetic polynucleotide
ttgtgcaattcgtgc

SEQ ID NO: 91 - DNA, 15 bp, Artificial Sequence
  Synthetic polynucleotide
ttgtgaaattggtgc

SEQ ID NO: 92 - DNA, 15 bp, Artificial Sequence
  Synthetic polynucleotide
ttgtccaattagtgc

SEQ ID NO: 93 - DNA, 10 bp, Artificial Sequence
  Synthetic polynucleotide
caatttgtgc